European Patent Specification EP 3 746 571 B1, published November 22, 2023. Title: Use of cfDNA fragments as biomarkers in patients. Applicant: Myway Genetics srl. The sequence listing filed with the application follows.

SEQUENCE LISTING (270 sequences)

SEQ ID NO: 1 - DNA, 26 bp, Homo sapiens
  source 1..26: /mol_type="other DNA" /organism="Homo sapiens"
tcagaccctagtcccagctgggtgag

SEQ ID NO: 2 - DNA, 27 bp, Homo sapiens
  source 1..27: /mol_type="other DNA" /organism="Homo sapiens"
ttgggggcatctgaaacactcacacac

SEQ ID NO: 3 - DNA, 23 bp, Homo sapiens
  source 1..23: /mol_type="other DNA" /organism="Homo sapiens"
ttccctggtcttgcccctgcact

SEQ ID NO: 4 - DNA, 27 bp, Homo sapiens
  source 1..27: /mol_type="other DNA" /organism="Homo sapiens"
caatgctcacagagatctcccagatca

SEQ ID NO: 5 - DNA, 27 bp, Homo sapiens
  source 1..27: /mol_type="other DNA" /organism="Homo sapiens"
gaatccacagctgcagaaaaccaaatg

SEQ ID NO: 6 - DNA, 30 bp, Homo sapiens
  source 1..30: /mol_type="other DNA" /organism="Homo sapiens"
tctatcacagaattatttatatatggccca

SEQ ID NO: 7 - DNA, 30 bp, Homo sapiens
  source 1..30: /mol_type="other DNA" /organism="Homo sapiens"
cgacatgggaaatgtcagatcataagacat

SEQ ID NO: 8 - DNA, 30 bp, Homo sapiens
  source 1..30: /mol_type="other DNA" /organism="Homo sapiens"
ctttggattctaaagtggatctaataacag

SEQ ID NO: 9 - DNA, 27 bp, Homo sapiens
  source 1..27: /mol_type="other DNA" /organism="Homo sapiens"
agcatttaaacagctatgaatccacct

SEQ ID NO: 10 - DNA, 27 bp, Homo sapiens
  source 1..27: /mol_type="other DNA" /organism="Homo sapiens"
tttcaacatgcccttagggaattcatg

SEQ ID NO: 11 - DNA, 27 bp, Homo sapiens
  source 1..27: /mol_type="other DNA" /organism="Homo sapiens"
caataacgtccagggagtgaaaaatcc

SEQ ID NO: 12 - DNA, 25 bp, Homo sapiens
  source 1..25: /mol_type="other DNA" /organism="Homo sapiens"
tacatgttccacttcccatgtgctc

SEQ ID NO: 13 - DNA, 27 bp, Homo sapiens
  source 1..27: /mol_type="other DNA" /organism="Homo sapiens"
tcaccagccccagcaagggcatgggga

SEQ ID NO: 14 - DNA, 23 bp, Homo sapiens
  source 1..23: /mol_type="other DNA" /organism="Homo sapiens"
aagaccacaggtcagggaggcat

SEQ ID NO: 15 - DNA, 28 bp, Homo sapiens
  source 1..28: /mol_type="other DNA" /organism="Homo sapiens"
ccaagccctatgccaaggatataacaat

SEQ ID NO: 16 - DNA, 27 bp, Homo sapiens
  source 1..27: /mol_type="other DNA" /organism="Homo sapiens"
atgggctcacggaagaagaacacaaag

SEQ ID NO: 17 - DNA, 28 bp, Homo sapiens
  source 1..28: /mol_type="other DNA" /organism="Homo sapiens"
gagcatacttgaaagcagtgattatatc

SEQ ID NO: 18 - DNA, 30 bp, Homo sapiens
  source 1..30: /mol_type="other DNA" /organism="Homo sapiens"
agacaaaaactggaaaatatttgaattacc

SEQ ID NO: 19 - DNA, 27 bp, Homo sapiens
  source 1..27: /mol_type="other DNA" /organism="Homo sapiens"
aagggtactcattaaccaagtgtttta

SEQ ID NO: 20 - DNA, 26 bp, Homo sapiens
  source 1..26: /mol_type="other DNA" /organism="Homo sapiens"
tctgaagcatgtttcgcaaagtgcag

SEQ ID NO: 21 - DNA, 27 bp, Homo sapiens
  source 1..27: /mol_type="other DNA" /organism="Homo sapiens"
gggaactcctaatacagtaaaacctct

SEQ ID NO: 22 - DNA, 28 bp, Homo sapiens
  source 1..28: /mol_type="other DNA" /organism="Homo sapiens"
cactagatttaagttctttcctgatgtg

SEQ ID NO: 23 - DNA, 27 bp, Homo sapiens
  source 1..27: /mol_type="other DNA" /organism="Homo sapiens"
gttctcccaaatttacattgccactga

SEQ ID NO: 24 - DNA, 27 bp, Homo sapiens
  source 1..27: /mol_type="other DNA" /organism="Homo sapiens"
caaggataccaaacctgcaggcataaa

SEQ ID NO: 25 - DNA, 24 bp, Homo sapiens
  source 1..24: /mol_type="other DNA" /organism="Homo sapiens"
atgccaggccagccacagagtgcc

SEQ ID NO: 26 - DNA, 26 bp, Homo sapiens
  source 1..26: /mol_type="other DNA" /organism="Homo sapiens"
cagaaccttgaaccagtgcatggtta

SEQ ID NO: 27 - DNA, 26 bp, Homo sapiens
  source 1..26: /mol_type="other DNA" /organism="Homo sapiens"
atcactgtccatcacgacaccgagtg

SEQ ID NO: 28 - DNA, 21 bp, Homo sapiens
  source 1..21: /mol_type="other DNA" /organism="Homo sapiens"
ccctccagtgttttgggtggg

SEQ ID NO: 29 - DNA, 26 bp, Homo sapiens
  source 1..26: /mol_type="other DNA" /organism="Homo sapiens"
tatgaacccccagcatggggcggggc

SEQ ID NO: 30 - DNA, 27 bp, Homo sapiens
  source 1..27: /mol_type="other DNA" /organism="Homo sapiens"
tctctctgggatcatgtgaggcgggaa

SEQ ID NO: 31 - DNA, 23 bp, Homo sapiens
  source 1..23: /mol_type="other DNA" /organism="Homo sapiens"
gggctgaaagatgatggcagagc

SEQ ID NO: 32 - DNA, 22 bp, Homo sapiens
  source 1..22: /mol_type="other DNA" /organism="Homo sapiens"
cctcaccaccagctctgtgaca

SEQ ID NO: 33 - DNA, 27 bp, Homo sapiens
  source 1..27: /mol_type="other DNA" /organism="Homo sapiens"
ggacaggtgcttggatgtcagggtgaa

SEQ ID NO: 34 - DNA, 27 bp, Homo sapiens
  source 1..27: /mol_type="other DNA" /organism="Homo sapiens"
gtccaaccaacaaggatgtggaggaat

SEQ ID NO: 35 - DNA, 26 bp, Homo sapiens
  source 1..26: /mol_type="other DNA" /organism="Homo sapiens"
ctggggatgaactctctttggagttt

SEQ ID NO: 36 - DNA, 27 bp, Homo sapiens
  source 1..27: /mol_type="other DNA" /organism="Homo sapiens"
tttggaagggtttttcgtcttgtttag

SEQ ID NO: 37 - DNA, 28 bp, Homo sapiens
  source 1..28: /mol_type="other DNA" /organism="Homo sapiens"
tcatttttaccatttaacagctctgatg

SEQ ID NO: 38 - DNA, 27 bp, Homo sapiens
  source 1..27: /mol_type="other DNA" /organism="Homo sapiens"
agaatcacagactcttacaggtcctag

SEQ ID NO: 39 - DNA, 27 bp, Homo sapiens
  source 1..27: /mol_type="other DNA" /organism="Homo sapiens"
tgagtttttacctacctttcttgcaca

SEQ ID NO: 40 - DNA, 27 bp, Homo sapiens
  source 1..27: /mol_type="other DNA" /organism="Homo sapiens"
agtgccttaacaacagcaaaatctctc

SEQ ID NO: 41 - DNA, 24 bp, Homo sapiens
  source 1..24: /mol_type="other DNA" /organism="Homo sapiens"
taccatgtctccccaggctctccg

SEQ ID NO: 42 - DNA, 29 bp, Homo sapiens
  source 1..29: /mol_type="other DNA" /organism="Homo sapiens"
ctccttaaaacatagtctgatacttatcg

SEQ ID NO: 43 - DNA, 27 bp, Homo sapiens
  source 1..27: /mol_type="other DNA" /organism="Homo sapiens"
aggtgggacaaaggcaggaagaaagta

SEQ ID NO: 44 - DNA, 27 bp, Homo sapiens
  source 1..27: /mol_type="other DNA" /organism="Homo sapiens"
ggcacacttaattttaacagaaggagg

SEQ ID NO: 45 - DNA, 27 bp, Homo sapiens
  source 1..27: /mol_type="other DNA" /organism="Homo sapiens"
cacagagacatgaggcattttcatgga

SEQ ID NO: 46 - DNA, 27 bp, Homo sapiens
  source 1..27: /mol_type="other DNA" /organism="Homo sapiens"
gtttcagtccacagcagaaaaagactc

SEQ ID NO: 47 - DNA, 27 bp, Homo sapiens
  source 1..27: /mol_type="other DNA" /organism="Homo sapiens"
gaggtacagctcccactgcctctgagt

SEQ ID NO: 48 - DNA, 27 bp, Homo sapiens
  source 1..27: /mol_type="other DNA" /organism="Homo sapiens"
ttgcccttttcattggacaactaaaaa

SEQ ID NO: 49 - DNA, 27 bp, Homo sapiens
  source 1..27: /mol_type="other DNA" /organism="Homo sapiens"
ctactgcacgtggatgatatggtttct

SEQ ID NO: 50 - DNA, 27 bp, Homo sapiens
  source 1..27: /mol_type="other DNA" /organism="Homo sapiens"
atgacattcatcaaaatgaaattgcca

SEQ ID NO: 51 - DNA, 27 bp, Homo sapiens
  source 1..27: /mol_type="other DNA" /organism="Homo sapiens"
aacaatacatacctgcaccctgccctt

SEQ ID NO: 52 - DNA, 27 bp, Homo sapiens
  source 1..27: /mol_type="other DNA" /organism="Homo sapiens"
gagagtgacatctaggttgtcatctga

SEQ ID NO: 53 - DNA, 29 bp, Homo sapiens
  source 1..29: /mol_type="other DNA" /organism="Homo sapiens"
ttgaaaaagcatcagattaaaacaaagat

SEQ ID NO: 54 - DNA, 27 bp, Homo sapiens
  source 1..27: /mol_type="other DNA" /organism="Homo sapiens"
agttcagcaaacactatgcaggataaa

SEQ ID NO: 55 - DNA, 27 bp, Homo sapiens
  source 1..27: /mol_type="other DNA" /organism="Homo sapiens"
cctttctgttttgtccatctgaaattc

SEQ ID NO: 56 - DNA, 29 bp, Homo sapiens
  source 1..29: /mol_type="other DNA" /organism="Homo sapiens"
taatgaaacatctgagtactttttaggtc

SEQ ID NO: 57 - DNA, 28 bp, Homo sapiens
  source 1..28: /mol_type="other DNA" /organism="Homo sapiens"
gtgtcttaaaacccatgattttcttgtg

SEQ ID NO: 58 - DNA, 27 bp, Homo sapiens
  source 1..27: /mol_type="other DNA" /organism="Homo sapiens"
attttccttcttcttgcagctttgagt

SEQ ID NO: 59 - DNA, 27 bp, Homo sapiens
  source 1..27: /mol_type="other DNA" /organism="Homo sapiens"
aggcctccagtggctctgaaattctca

SEQ ID NO: 60 - DNA, 27 bp, Homo sapiens
  source 1..27: /mol_type="other DNA" /organism="Homo sapiens"
tcttcagacctgtaatggggctatttg

SEQ ID NO: 61 - DNA, 26 bp, Homo sapiens
  source 1..26: /mol_type="other DNA" /organism="Homo sapiens"
cagaccacttcaccctctgtacttta

SEQ ID NO: 62 - DNA, 23 bp, Homo sapiens
  source 1..23: /mol_type="other DNA" /organism="Homo sapiens"
gtttgagacacaattcccccagg

SEQ ID NO: 63 - DNA, 25 bp, Homo sapiens
  source 1..25: /mol_type="other DNA" /organism="Homo sapiens"
cccaaattcagcttgggaagtcaaa

SEQ ID NO: 64 - DNA, 27 bp, Homo sapiens
  source 1..27: /mol_type="other DNA" /organism="Homo sapiens"
agattttgctgtgaaagtgagtgtctg

SEQ ID NO: 65 - DNA, 25 bp, Homo sapiens
  source 1..25: /mol_type="other DNA" /organism="Homo sapiens"
gtcacagcttcgctttgctactctt

SEQ ID NO: 66 - DNA, 20 bp, Homo sapiens
  source 1..20: /mol_type="other DNA" /organism="Homo sapiens"
gacggcaggtgggggtcacc

SEQ ID NO: 67 - DNA, 27 bp, Homo sapiens
  source 1..27: /mol_type="other DNA" /organism="Homo sapiens"
cctccagacctgaaagatggaggcttt

SEQ ID NO: 68 - DNA, 27 bp, Homo sapiens
  source 1..27: /mol_type="other DNA" /organism="Homo sapiens"
gtgtccccctcaatcccctctccattt

SEQ ID NO: 69 - DNA, 29 bp, Homo sapiens
  source 1..29: /mol_type="other DNA" /organism="Homo sapiens"
tgtagaatttgattaaagtgtcttctgga

SEQ ID NO: 70 - DNA, 29 bp, Homo sapiens
  source 1..29: /mol_type="other DNA" /organism="Homo sapiens"
gctctgtaacatcctaagggatttttgct

SEQ ID NO: 71 - DNA, 27 bp, Homo sapiens
  source 1..27: /mol_type="other DNA" /organism="Homo sapiens"
gccgacttattagacggacagcatttt

SEQ ID NO: 72 - DNA, 27 bp, Homo sapiens
  source 1..27: /mol_type="other DNA" /organism="Homo sapiens"
aatggaatgttgcagcttgaacataat

SEQ ID NO: 73 - DNA, 27 bp, Homo sapiens
  source 1..27: /mol_type="other DNA" /organism="Homo sapiens"
ctggaacacatcaaaaaccaccatctc

SEQ ID NO: 74 - DNA, 23 bp, Homo sapiens
  source 1..23: /mol_type="other DNA" /organism="Homo sapiens"
gcctcacccaaaggcagacatag

SEQ ID NO: 75 - DNA, 26 bp, Homo sapiens
  source 1..26: /mol_type="other DNA" /organism="Homo sapiens"
atacttggctgtctgggagcctgtag

SEQ ID NO: 76 - DNA, 26 bp, Homo sapiens
  source 1..26: /mol_type="other DNA" /organism="Homo sapiens"
atgggcatacatgcatacacatgtgc

SEQ ID NO: 77 - DNA, 27 bp, Homo sapiens
  source 1..27: /mol_type="other DNA" /organism="Homo sapiens"
atgttggtggaagggactgagaagcct

SEQ ID NO: 78 - DNA, 27 bp, Homo sapiens
  source 1..27: /mol_type="other DNA" /organism="Homo sapiens"
tttctgtgctgagcattttatatgtgc

SEQ ID NO: 79 - DNA, 27 bp, Homo sapiens
  source 1..27: /mol_type="other DNA" /organism="Homo sapiens"
tcacagtgatccatacactaaaacaag

SEQ ID NO: 80 - DNA, 30 bp, Homo sapiens
  source 1..30: /mol_type="other DNA" /organism="Homo sapiens"
agacttttgttaaattatcatcaaggagat

SEQ ID NO: 81 - DNA, 27 bp, Homo sapiens
  source 1..27: /mol_type="other DNA" /organism="Homo sapiens"
ccagagacctgttctctgtccattatt

SEQ ID NO: 82 - DNA, 27 bp, Homo sapiens
  source 1..27: /mol_type="other DNA" /organism="Homo sapiens"
aattgcagctgagagaaaacagtagta

SEQ ID NO: 83 - DNA, 27 bp, Homo sapiens
  source 1..27: /mol_type="other DNA" /organism="Homo sapiens"
gatctatggaagtgctgagaagggaag

SEQ ID NO: 84 - DNA, 27 bp, Homo sapiens
  source 1..27: /mol_type="other DNA" /organism="Homo sapiens"
cgctcactcccctacaaatgtcaacaa

SEQ ID NO: 85 - DNA, 24 bp, Homo sapiens
  source 1..24: /mol_type="other DNA" /organism="Homo sapiens"
tgggtgagacaatgcacagaactg

SEQ ID NO: 86 - DNA, 26 bp, Homo sapiens
  source 1..26: /mol_type="other DNA" /organism="Homo sapiens"
aaaaagcactgggatcctcactttgg

SEQ ID NO: 87 - DNA, 27 bp, Homo sapiens
  source 1..27: /mol_type="other DNA" /organism="Homo sapiens"
gatgctatcgctggctattaggtgatc

SEQ ID NO: 88 - DNA, 27 bp, Homo sapiens
  source 1..27: /mol_type="other DNA" /organism="Homo sapiens"
atacaggtagagagtgatgaagccaag

SEQ ID NO: 89 - DNA, 27 bp, Homo sapiens
  source 1..27: /mol_type="other DNA" /organism="Homo sapiens"
agagagattgattatgttgggatgggg

SEQ ID NO: 90 - DNA, 26 bp, Homo sapiens
  source 1..26: /mol_type="other DNA" /organism="Homo sapiens"
tgcagtttgctgagtttcaccaaatc

SEQ ID NO: 91 - DNA, 27 bp, Homo sapiens
  source 1..27: /mol_type="other DNA" /organism="Homo sapiens"
tgatccacattgtatggtttttaggca

SEQ ID NO: 92 - DNA, 27 bp, Homo sapiens
  source 1..27: /mol_type="other DNA" /organism="Homo sapiens"
gtgcttattagatgtttgtgctcacaa

SEQ ID NO: 93 - DNA, 27 bp, Homo sapiens
  source 1..27: /mol_type="other DNA" /organism="Homo sapiens"
ttgatgtttctgtgtgttgagtggggg

SEQ ID NO: 94 - DNA, 27 bp, Homo sapiens
  source 1..27: /mol_type="other DNA" /organism="Homo sapiens"
ggatctggctgttccttagttcatcat

SEQ ID NO: 95 - DNA, 23 bp, Homo sapiens
  source 1..23: /mol_type="other DNA" /organism="Homo sapiens"
agagcgcttgtctgaatggagac

SEQ ID NO: 96 - DNA, 27 bp, Homo sapiens
  source 1..27: /mol_type="other DNA" /organism="Homo sapiens"
cattttaaagaaaagaggagctgggtg

SEQ ID NO: 97 - DNA, 27 bp, Homo sapiens
  source 1..27: /mol_type="other DNA" /organism="Homo sapiens"
cagtgcaagacaagcgattgaaagaag

SEQ ID NO: 98 - DNA, 26 bp, Homo sapiens
  source 1..26: /mol_type="other DNA" /organism="Homo sapiens"
aagggacaaggaaagagtgctccttc

SEQ ID NO: 99 - DNA, 27 bp, Homo sapiens
  source 1..27: /mol_type="other DNA" /organism="Homo sapiens"
cccagtctccaaaccgctgtaatattt

SEQ ID NO: 100 - DNA, 24 bp, Homo sapiens
  source 1..24: /mol_type="other DNA" /organism="Homo sapiens"
gcccttgtgcacatagatgcaaag

SEQ ID NO: 101 - DNA, 26 bp, Homo sapiens
  source 1..26: /mol_type="other DNA" /organism="Homo sapiens"
atgagcaagagttccaacgttccatg

SEQ ID NO: 102 - DNA, 27 bp, Homo sapiens
  source 1..27: /mol_type="other DNA" /organism="Homo sapiens"
tgaatccaaaggtggattctctaaggc

SEQ ID NO: 103 - DNA, 29 bp, Homo sapiens
  source 1..29: /mol_type="other DNA" /organism="Homo sapiens"
aaattgaatcatagcttgtgttggtcagg

SEQ ID NO: 104 - DNA, 29 bp, Homo sapiens
  source 1..29: /mol_type="other DNA" /organism="Homo sapiens"
ttctcaaaggaaagaaaaatatcagttca

SEQ ID NO: 105 - DNA, 27 bp, Homo sapiens
  source 1..27: /mol_type="other DNA" /organism="Homo sapiens"
cagaccaacttggctttaacagatgca

SEQ ID NO: 106 - DNA, 26 bp, Homo sapiens
  source 1..26: /mol_type="other DNA" /organism="Homo sapiens"
cacaaaagaactggcattccagaact

SEQ ID NO: 107 - DNA, 29 bp, Homo sapiens
  source 1..29: /mol_type="other DNA" /organism="Homo sapiens"
tgtatccttacctttaagacttttcctat

SEQ ID NO: 108 - DNA, 27 bp, Homo sapiens
  source 1..27: /mol_type="other DNA" /organism="Homo sapiens"
atgcaaatatcagttttgatgaagcaa

SEQ ID NO: 109 - DNA, 29 bp, Homo sapiens
  source 1..29: /mol_type="other DNA" /organism="Homo sapiens"
tgatcgttcatagacaatagatacataca

SEQ ID NO: 110 - DNA, 24 bp, Homo sapiens
  source 1..24: /mol_type="other DNA" /organism="Homo sapiens"
ggctttcaagcgtttctgcaatga

SEQ ID NO: 111 - RNA, 27 nt, Homo sapiens
  source 1..27: /mol_type="transcribed RNA" /organism="Homo sapiens"
cgttctgtataggcaccatatagcact

SEQ ID NO: 112 - DNA, 24 bp, Homo sapiens
  source 1..24: /mol_type="other DNA" /organism="Homo sapiens"
acggattgaatgaagcagcggtct

SEQ ID NO: 113 - DNA, 27 bp, Homo sapiens
  source 1..27: /mol_type="other DNA" /organism="Homo sapiens"
agacttttggcttaaatcaatgggtct

SEQ ID NO: 114 - DNA, 27 bp, Homo sapiens
  source 1..27: /mol_type="other DNA" /organism="Homo sapiens"
tcatgggagtttctgatgtcactaagg

SEQ ID NO: 115 - DNA, 28 bp, Homo sapiens
  source 1..28: /mol_type="other DNA" /organism="Homo sapiens"
accactcacatgtcaaataaaataactg

SEQ ID NO: 116 - DNA, 29 bp, Homo sapiens
  source 1..29: /mol_type="other DNA" /organism="Homo sapiens"
ctcccactgaacttcataaaaacaaaaga

SEQ ID NO: 117 - DNA, 27 bp, Homo sapiens
  source 1..27: /mol_type="other DNA" /organism="Homo sapiens"
ttatccctttcctgtctgggctgaatc

SEQ ID NO: 118 - DNA, 20 bp, Homo sapiens
  source 1..20: /mol_type="other DNA" /organism="Homo sapiens"
gggggttggagtggggcgga

SEQ ID NO: 119 - DNA, 27 bp, Homo sapiens
  source 1..27: /mol_type="other DNA" /organism="Homo sapiens"
gtgcacattctaagaactggtgattct

SEQ ID NO: 120 - DNA, 23 bp, Homo sapiens
  source 1..23: /mol_type="other DNA" /organism="Homo sapiens"
ccttcagggatttccagcagtgg

SEQ ID NO: 121 - DNA, 27 bp, Homo sapiens
  source 1..27: /mol_type="other DNA" /organism="Homo sapiens"
tttggagcttggtgatgagtggaggct

SEQ ID NO: 122 - DNA, 26 bp, Homo sapiens
  source 1..26: /mol_type="other DNA" /organism="Homo sapiens"
agacaaccatgagcagaatgctggta

SEQ ID NO: 123 - DNA, 26 bp, Homo sapiens
  source 1..26: /mol_type="other DNA" /organism="Homo sapiens"
ttctgttgtggctcgtcttcctgagc

SEQ ID NO: 124 - DNA, 21 bp, Homo sapiens
  source 1..21: /mol_type="other DNA" /organism="Homo sapiens"
gcctctgagagggtagggaca

SEQ ID NO: 125 - DNA, 27 bp, Homo sapiens
  source 1..27: /mol_type="other DNA" /organism="Homo sapiens"
atccaatgctcaggggagacattagct

SEQ ID NO: 126 - DNA, 30 bp, Homo sapiens
  source 1..30: /mol_type="other DNA" /organism="Homo sapiens"
tcctatctaattcttctaatttctcgtcaa

SEQ ID NO: 127 - DNA, 27 bp, Homo sapiens
  source 1..27: /mol_type="other DNA" /organism="Homo sapiens"
ccagcatctgttgttttaactttcttt

SEQ ID NO: 128 - DNA, 28 bp, Homo sapiens
  source 1..28: /mol_type="other DNA" /organism="Homo sapiens"
agaagtatctgttcatgtattttgctga

SEQ ID NO: 129 - DNA, 26 bp, Homo sapiens
  source 1..26: /mol_type="other DNA" /organism="Homo sapiens"
caaagaactgacccttgcagagaact

SEQ ID NO: 130 - DNA, 26 bp, Homo sapiens
  source 1..26: /mol_type="other DNA" /organism="Homo sapiens"
gattctagcaagagaatgcaggtgct

SEQ ID NO: 131 - DNA, 28 bp, Homo sapiens
  source 1..28: /mol_type="other DNA" /organism="Homo sapiens"
actccagaagctactgggatattaatta

SEQ ID NO: 132 - DNA, 28 bp, Homo sapiens
  source 1..28: /mol_type="other DNA" /organism="Homo sapiens"
gttcattaagaaaacctgtgacaaacat

SEQ ID NO: 133 - DNA, 30 bp, Homo sapiens
  source 1..30: /mol_type="other DNA" /organism="Homo sapiens"
tctctaaacttccttgatattaactactga

SEQ ID NO: 134 - DNA, 27 bp, Homo sapiens
  source 1..27: /mol_type="other DNA" /organism="Homo sapiens"
atacttaccagactgcctgcttcttag

SEQ ID NO: 135 - DNA, 27 bp, Homo sapiens
  source 1..27: /mol_type="other DNA" /organism="Homo sapiens"
gaacatagttcaaggaggtacagcctc

SEQ ID NO: 136 - DNA, 25 bp, Homo sapiens
  source 1..25: /mol_type="other DNA" /organism="Homo sapiens"
tgcagccttcctatttaccgaaagc

SEQ ID NO: 137 - DNA, 27 bp, Homo sapiens
  source 1..27: /mol_type="other DNA" /organism="Homo sapiens"
cagtctgtgtagccaacacacactaat

SEQ ID NO: 138 - DNA, 27 bp, Homo sapiens
  source 1..27: /mol_type="other DNA" /organism="Homo sapiens"
ccaatttcccagcctacatcagctatt

SEQ ID NO: 139 - DNA, 27 bp, Homo sapiens
  source 1..27: /mol_type="other DNA" /organism="Homo sapiens"
taaacctattccactaacttcaggaac

SEQ ID NO: 140 - DNA, 27 bp, Homo sapiens
  source 1..27: /mol_type="other DNA" /organism="Homo sapiens"
agtgtacctgcagaactgtagagaatc

SEQ ID NO: 141 - DNA, 27 bp, Homo sapiens
  source 1..27: /mol_type="other DNA" /organism="Homo sapiens"
cagaagtggaatcacaaaaggaaaaca

SEQ ID NO: 142 - DNA, 27 bp, Homo sapiens
  source 1..27: /mol_type="other DNA" /organism="Homo sapiens"
aaattgtaggtgtgtaagtgcatctct

SEQ ID NO: 143 - DNA, 25 bp, Homo sapiens
  source 1..25: /mol_type="other DNA" /organism="Homo sapiens"
ctcctacacacaggcttcaggttac

SEQ ID NO: 144 - DNA, 26 bp, Homo sapiens
  source 1..26: /mol_type="other DNA" /organism="Homo sapiens"
atttttcccagtccctttaccaaaaa

SEQ ID NO: 145 - DNA, 25 bp, Homo sapiens
  source 1..25: /mol_type="other DNA" /organism="Homo sapiens"
tgtgcctgtgcacacacacgtttgg

SEQ ID NO: 146 - DNA, 20 bp, Homo sapiens
  source 1..20: /mol_type="other DNA" /organism="Homo sapiens"
gccaggagcgcagctcacgc

SEQ ID NO: 147 - DNA, 23 bp, Homo sapiens
  source 1..23: /mol_type="other DNA" /organism="Homo sapiens"
cagccgaagaatccagcccttgt

SEQ ID NO: 148 - DNA, 27 bp, Homo sapiens
  source 1..27: /mol_type="other DNA" /organism="Homo sapiens"
gacctttccccgctcagagctccttca

SEQ ID NO: 149 - DNA, 28 bp, Homo sapiens
  source 1..28: /mol_type="other DNA" /organism="Homo sapiens"
aaagaggggtgttctggtggcttctctt

SEQ ID NO: 150 - DNA, 25 bp, Homo sapiens
  source 1..25: /mol_type="other DNA" /organism="Homo sapiens"
cacctcttatcagtacgcaggcaaa

SEQ ID NO: 151 - DNA, 27 bp, Homo sapiens
  source 1..27: /mol_type="other DNA" /organism="Homo sapiens"
gtgatacatgagagagatacataaggg

SEQ ID NO: 152 - DNA, 26 bp, Homo sapiens
  source 1..26: /mol_type="other DNA" /organism="Homo sapiens"
tcctccctgaaaattatagcaggtct

SEQ ID NO: 153 - DNA, 26 bp, Homo sapiens
  source 1..26: /mol_type="other DNA" /organism="Homo sapiens"
acgggtgaaagctgatatcttgacct

SEQ ID NO: 154 - DNA, 27 bp, Homo sapiens
  source 1..27: /mol_type="other DNA" /organism="Homo sapiens"
gtaatttgccatcactttcagtggcaa

SEQ ID NO: 155 - DNA, 27 bp, Homo sapiens
  source 1..27: /mol_type="other DNA" /organism="Homo sapiens"
tcaaaaacaaagaaacatgggatgaac

SEQ ID NO: 156 - DNA, 27 bp, Homo sapiens
  source 1..27: /mol_type="other DNA" /organism="Homo sapiens"
cagatccatcattgccagtagacaaac

SEQ ID NO: 157 - DNA, 25 bp, Homo sapiens
  source 1..25: /mol_type="other DNA" /organism="Homo sapiens"
caagaggagtcaaggcatttgacca

SEQ ID NO: 158 - DNA, 22 bp, Homo sapiens
  source 1..22: /mol_type="other DNA" /organism="Homo sapiens"
ttggcattcagcggcccccaga

SEQ ID NO: 159 - DNA, 27 bp, Homo sapiens
  source 1..27: /mol_type="other DNA" /organism="Homo sapiens"
cattcaccatttgatagccatttgggt

SEQ ID NO: 160 - DNA, 30 bp, Homo sapiens
  source 1..30: /mol_type="other DNA" /organism="Homo sapiens"
tgtaagtaattataccattttacactccca

SEQ ID NO: 161 - DNA, 26 bp, Homo sapiens
  source 1..26: /mol_type="other DNA" /organism="Homo sapiens"
gttttgatcaccaaccacttgcagtt

SEQ ID NO: 162 - DNA, 30 bp, Homo sapiens
  source 1..30: /mol_type="other DNA" /organism="Homo sapiens"
gcctggacaacatgatgtctctatattaaa

SEQ ID NO: 163 - DNA, 27 bp, Homo sapiens
  source 1..27: /mol_type="other DNA" /organism="Homo sapiens"
cacctggcctacaattcaaattaatgt

SEQ ID NO: 164 - DNA, 29 bp, Homo sapiens
  source 1..29: /mol_type="other DNA" /organism="Homo sapiens"
agtttgaatcagaaataagatgtgaatga

SEQ ID NO: 165 - DNA, 24 bp, Homo sapiens
  source 1..24: /mol_type="other DNA" /organism="Homo sapiens"
actcctggggatacaagagcttcc

SEQ ID NO: 166 - DNA, 27 bp, Homo sapiens
  source 1..27: /mol_type="other DNA" /organism="Homo sapiens"
ttattgtcagcgttgtttaaattctgg

SEQ ID NO: 167 - DNA, 21 bp, Homo sapiens
  source 1..21: /mol_type="other DNA" /organism="Homo sapiens"
gaggaagccgttgctggtctc

SEQ ID NO: 168 - DNA, 26 bp, Homo sapiens
  source 1..26: /mol_type="other DNA" /organism="Homo sapiens"
atctccaagctcagctcagcccaaga

SEQ ID NO: 169 - DNA, 24 bp, Homo sapiens
  source 1..24: /mol_type="other DNA" /organism="Homo sapiens"
aatctgagctcgaggtagcaggaa

SEQ ID NO: 170 - DNA, 21 bp, Homo sapiens
  source 1..21: /mol_type="other DNA" /organism="Homo sapiens"
cagggagggctttggtgtctg

SEQ ID NO: 171 - DNA, 27 bp, Homo sapiens
  source 1..27: /mol_type="other DNA" /organism="Homo sapiens"
ggcctgtgctttcactgggatgcaaat

SEQ ID NO: 172 - DNA, 26 bp, Homo sapiens
  source 1..26: /mol_type="other DNA" /organism="Homo sapiens"
gtggggaaaagtgagtgattcgtgtt

SEQ ID NO: 173 - DNA, 27 bp, Homo sapiens
  source 1..27: /mol_type="other DNA" /organism="Homo sapiens"
cgtgactctcatatatctgtggaagca

SEQ ID NO: 174 - DNA, 25 bp, Homo sapiens
  source 1..25: /mol_type="other DNA" /organism="Homo sapiens"
tcagaaagaaactggtgggaactcc

SEQ ID NO: 175 - DNA, 27 bp, Homo sapiens
  source 1..27: /mol_type="other DNA" /organism="Homo sapiens"
aggcatttttctctcatcttgtttgca

SEQ ID NO: 176 - DNA, 23 bp, Homo sapiens
  source 1..23: /mol_type="other DNA" /organism="Homo sapiens"
gggaggcacaaaagaggttgatg

SEQ ID NO: 177 - DNA, 28 bp, Homo sapiens
  source 1..28: /mol_type="other DNA" /organism="Homo sapiens"
gttagaaaggagaatcaggaaatagtca

SEQ ID NO: 178 - DNA, 30 bp, Homo sapiens
  source 1..30: /mol_type="other DNA" /organism="Homo sapiens"
cctctttaatttactcaagactaattagcc

SEQ ID NO: 179 - DNA, 23 bp, Homo sapiens
  source 1..23: /mol_type="other DNA" /organism="Homo sapiens"
tcaaagcaccaggcatttgacct

SEQ ID NO: 180 - DNA, 27 bp, Homo sapiens
  source 1..27: /mol_type="other DNA" /organism="Homo sapiens"
gggataaatttggcctctgtatcaacc

SEQ ID NO: 181 - DNA, 29 bp, Homo sapiens
  source 1..29: /mol_type="other DNA" /organism="Homo sapiens"
attttcatagaagtacttcatttggctag

SEQ ID NO: 182 - DNA, 27 bp, Homo sapiens
  source 1..27: /mol_type="other DNA" /organism="Homo sapiens"
ttcccaactatggtgaaagaaaatcaa

SEQ ID NO: 183 - DNA, 27 bp, Homo sapiens
  source 1..27: /mol_type="other DNA" /organism="Homo sapiens"
ttcttatgtaatcgtcatccaacaaga

SEQ ID NO: 184 - DNA, 27 bp, Homo sapiens
  source 1..27: /mol_type="other DNA" /organism="Homo sapiens"
ggagaggatggtgtggggaaaataaaa

SEQ ID NO: 185 - DNA, 27 bp, Homo sapiens
  source 1..27: /mol_type="other DNA" /organism="Homo sapiens"
gaaatactttccccaacaaggcagttt

SEQ ID NO: 186 - DNA, 27 bp, Homo sapiens
  source 1..27: /mol_type="other DNA" /organism="Homo sapiens"
tgacaaaataacaagttccgtttgatt

SEQ ID NO: 187 - DNA, 28 bp, Homo sapiens
  source 1..28: /mol_type="other DNA" /organism="Homo sapiens"
cgttcaccacacagttaatacgatatgc

SEQ ID NO: 188 - DNA, 27 bp, Homo sapiens
  source 1..27: /mol_type="other DNA" /organism="Homo sapiens"
tctctagaacctgccaaatcacttatt

SEQ ID NO: 189 - DNA, 30 bp, Homo sapiens
  source 1..30: /mol_type="other DNA" /organism="Homo sapiens"
ataaaaggatatggcaaataagctttagaa

SEQ ID NO: 190 - DNA, 27 bp, Homo sapiens
  source 1..27: /mol_type="other DNA" /organism="Homo sapiens"
gattgcttgcccacattccattcaaag

SEQ ID NO: 191 - DNA, 27 bp, Homo sapiens
  source 1..27: /mol_type="other DNA" /organism="Homo sapiens"
gattgcttgcccacattccattcaaag

SEQ ID NO: 192 - DNA, 27 bp, Homo sapiens
  source 1..27: /mol_type="other DNA" /organism="Homo sapiens"
gattgcttgcccacattccattcaaag

SEQ ID NO: 193 - DNA, 27 bp, Homo sapiens
  source 1..27: /mol_type="other DNA" /organism="Homo sapiens"
gattgcttgcccacattccattcaaag

SEQ ID NO: 194 - DNA, 27 bp, Homo sapiens
  source 1..27: /mol_type="other DNA" /organism="Homo sapiens"
gattgcttgcccacattccattcaaag

SEQ ID NO: 195 - DNA, 27 bp, Homo sapiens
  source 1..27: /mol_type="other DNA" /organism="Homo sapiens"
gattgcttgcccacattccattcaaag

SEQ ID NO: 196 - DNA, 27 bp, Homo sapiens
  source 1..27: /mol_type="other DNA" /organism="Homo sapiens"
gattgcttgcccacattccattcaaag

SEQ ID NO: 197 - DNA, 27 bp, Homo sapiens
  source 1..27: /mol_type="other DNA" /organism="Homo sapiens"
gattgcttgcccacattccattcaaag

SEQ ID NO: 198 - DNA, 27 bp, Homo sapiens
  source 1..27: /mol_type="other DNA" /organism="Homo sapiens"
gattgcttgcccacattccattcaaag

SEQ ID NO: 199 - DNA, 27 bp, Homo sapiens
  source 1..27: /mol_type="other DNA" /organism="Homo sapiens"
gattgcttgcccacattccattcaaag

SEQ ID NO: 200 - DNA, 27 bp, Homo sapiens
  source 1..27: /mol_type="other DNA" /organism="Homo sapiens"
gattgcttgcccacattccattcaaag

SEQ ID NO: 201 - DNA, 26 bp, Homo sapiens
  source 1..26: /mol_type="other DNA" /organism="Homo sapiens"
atgattgtaagtcgttgaagttccgg

SEQ ID NO: 202 - DNA, 27 bp, Homo sapiens
  source 1..27: /mol_type="other DNA" /organism="Homo sapiens"
aaagaacatactttggctcattctggt

SEQ ID NO: 203 - DNA, 27 bp, Homo sapiens
  source 1..27: /mol_type="other DNA" /organism="Homo sapiens"
ctgagatccctttgatagcgctttcta

SEQ ID NO: 204 - DNA, 30 bp, Homo sapiens
  source 1..30: /mol_type="other DNA" /organism="Homo sapiens"
catatttcctcaatataaattctaacacgc

SEQ ID NO: 205 - DNA, 26 bp, Homo sapiens
  source 1..26: /mol_type="other DNA" /organism="Homo sapiens"
taggggttgagtccatgccaagacaa

SEQ ID NO: 206 - DNA, 26 bp, Homo sapiens
  source 1..26: /mol_type="other DNA" /organism="Homo sapiens"
accacatccccaattagagtcaagaa

SEQ ID NO: 207 - DNA, 25 bp, Homo sapiens
  source 1..25: /mol_type="other DNA" /organism="Homo sapiens"
cttgccaaagaaaactcaagcgagg

SEQ ID NO: 208 - DNA, 27 bp, Homo sapiens
  source 1..27: /mol_type="other DNA" /organism="Homo sapiens"
gggggcacttctgaaggggactgtgtt

SEQ ID NO: 209 - DNA, 30 bp, Homo sapiens
  source 1..30: /mol_type="other DNA" /organism="Homo sapiens"
aaaaagaaggtcgacgccggctccagaagg

SEQ ID NO: 210 - DNA, 22 bp, Homo sapiens
  source 1..22: /mol_type="other DNA" /organism="Homo sapiens"
cgactagcccggtttcccaaga

SEQ ID NO: 211 - DNA, 25 bp, Homo sapiens
  source 1..25: /mol_type="other DNA" /organism="Homo sapiens"
ctctccggttttctccaggttaggt

SEQ ID NO: 212 - DNA, 27 bp, Homo sapiens
  source 1..27: /mol_type="other DNA" /organism="Homo sapiens"
gacagcaaaacatggacaaaccctatc

SEQ ID NO: 213 - DNA, 26 bp, Homo sapiens
  source 1..26: /mol_type="other DNA" /organism="Homo sapiens"
ttactgtgatgtaggcactgttccag

SEQ ID NO: 214 - DNA, 26 bp, Homo sapiens
  source 1..26: /mol_type="other DNA" /organism="Homo sapiens"
agagaggtctcagggcccaagccatc

SEQ ID NO: 215 - DNA, 26 bp, Homo sapiens
  source 1..26: /mol_type="other DNA" /organism="Homo sapiens"
attgtcctccttgagatgtggcttcc

SEQ ID NO: 216 - DNA, 27 bp, Homo sapiens
  source 1..27: /mol_type="other DNA" /organism="Homo sapiens"
ccattacctgagaaggcatttctaaag

SEQ ID NO: 217 - DNA, 27 bp, Homo sapiens
  source 1..27: /mol_type="other DNA" /organism="Homo sapiens"
ccggttcattaataagacgggacatcc

SEQ ID NO: 218 - DNA, 27 bp, Homo sapiens
  source 1..27: /mol_type="other DNA" /organism="Homo sapiens"
gggtttcatgttatggagaaaaacaac

SEQ ID NO: 219 - DNA, 27 bp, Homo sapiens
  source 1..27: /mol_type="other DNA" /organism="Homo sapiens"
ccctttctctgttcataggcaaacaca

SEQ ID NO: 220 - DNA, 27 bp, Homo sapiens
  source 1..27: /mol_type="other DNA" /organism="Homo sapiens"
tctaactcattctttttaacagctgcg

SEQ ID NO: 221 - DNA, 27 bp, Homo sapiens
  source 1..27: /mol_type="other DNA" /organism="Homo sapiens"
cagccaaaccatatcaagtgctttctg

SEQ ID NO: 222 - DNA, 29 bp, Homo sapiens
  source 1..29: /mol_type="other DNA" /organism="Homo sapiens"
tgtttgtaattgattttgttactctttgg

SEQ ID NO: 223 - DNA, 29 bp, Homo sapiens
  source 1..29: /mol_type="other DNA" /organism="Homo sapiens"
aaatgtatacattatttgctgaaaagtgc

SEQ ID NO: 224 - DNA, 27 bp, Homo sapiens
  source 1..27: /mol_type="other DNA" /organism="Homo sapiens"
tgataaatgttgaagcctacactgaag

SEQ ID NO: 225 - DNA, 24 bp, Homo sapiens
  source 1..24: /mol_type="other DNA" /organism="Homo sapiens"
aacctctgtgttctgagccacgtg

SEQ ID NO: 226 - DNA, 26 bp, Homo sapiens
  source 1..26: /mol_type="other DNA" /organism="Homo sapiens"
tagctgcttcagcctggtggtctggg

SEQ ID NO: 227 - DNA, 27 bp, Homo sapiens
  source 1..27: /mol_type="other DNA" /organism="Homo sapiens"
tccttgaggctcttctcacactcagat

SEQ ID NO: 228 - DNA, 27 bp, Homo sapiens
  source 1..27: /mol_type="other DNA" /organism="Homo sapiens"
aatatgactggagttcatctgtgtgcc

SEQ ID NO: 229 - DNA, 25 bp, Homo sapiens
  source 1..25: /mol_type="other DNA" /organism="Homo sapiens"
tctgctatcctgatgagagataggt

SEQ ID NO: 230 - DNA, 29 bp, Homo sapiens
  source 1..29: /mol_type="other DNA" /organism="Homo sapiens"
tttctcaaatacacaaaagagtttaccaa

SEQ ID NO: 231 - DNA, 30 bp, Homo sapiens
  source 1..30: /mol_type="other DNA" /organism="Homo sapiens"
tgatgctgaattttgtctctgttatattag

SEQ ID NO: 232 - DNA, 27 bp, Homo sapiens
  source 1..27: /mol_type="other DNA" /organism="Homo sapiens"
ttttcctcttgatccctcatattgcct

SEQ ID NO: 233 - DNA, 26 bp, Homo sapiens
  source 1..26: /mol_type="other DNA" /organism="Homo sapiens"
tctctctggttcacaaatgagcatgc

SEQ ID NO: 234 - DNA, 27 bp, Homo sapiens
  source 1..27: /mol_type="other DNA" /organism="Homo sapiens"
gctgccatttttcttccaggaagtatc

SEQ ID NO: 235 - DNA, 21 bp, Homo sapiens
  source 1..21: /mol_type="other DNA" /organism="Homo sapiens"
actccaactcctgccagcctt

SEQ ID NO: 236 - DNA, 26 bp, Homo sapiens
  source 1..26: /mol_type="other DNA" /organism="Homo sapiens"
ggccagcctgactaacatggcaaaat

SEQ ID NO: 237 - DNA, 30 bp, Homo sapiens
  source 1..30: /mol_type="other DNA" /organism="Homo sapiens"
gttgtttaaacattttaaaccatgagaagt

SEQ ID NO: 238 - DNA, 22 bp, Homo sapiens
  source 1..22: /mol_type="other DNA" /organism="Homo sapiens"
tgcatgatgattcccctgccaa

SEQ ID NO: 239 - DNA, 28 bp, Homo sapiens
  source 1..28: /mol_type="other DNA" /organism="Homo sapiens"
tcaaatttagtagatgtagacagactcc

SEQ ID NO: 240 - DNA, 30 bp, Homo sapiens
  source 1..30: /mol_type="other DNA" /organism="Homo sapiens"
gactgttctctggcttaagatttatttagg

SEQ ID NO: 241 - DNA, 30 bp, Homo sapiens
  source 1..30: /mol_type="other DNA" /organism="Homo sapiens"
cttgtgttttcttcaatcacttcttatttt

SEQ ID NO: 242 - DNA, 27 bp, Homo sapiens
  source 1..27: /mol_type="other DNA" /organism="Homo sapiens"
aagtgtacaaaactccatgtaccaggt

SEQ ID NO: 243 - DNA, 26 bp, Homo sapiens
  source 1..26: /mol_type="other DNA" /organism="Homo sapiens"
agaggcaacgccaccatcatacagac

SEQ ID NO: 244 - DNA, 26 bp, Homo sapiens
  source 1..26: /mol_type="other DNA" /organism="Homo sapiens"
atggctgtcctcctggatggtaaata

SEQ ID NO: 245 - DNA, 27 bp, Homo sapiens
  source 1..27: /mol_type="other DNA" /organism="Homo sapiens"
cgaaaaggtgaaaccagtcctcttttg

SEQ ID NO: 246 - DNA, 27 bp, Homo sapiens
  source 1..27: /mol_type="other DNA" /organism="Homo sapiens"
agaatcgttatcaggaactccctgggc

SEQ ID NO: 247 - DNA, 30 bp, Homo sapiens
  source 1..30: /mol_type="other DNA" /organism="Homo sapiens"
tataaatcacggagtgcagaccagtcacct

SEQ ID NO: 248 - DNA, 27 bp, Homo sapiens
  source 1..27: /mol_type="other DNA" /organism="Homo sapiens"
agggtcccgtgtgatcatcattgtatc

SEQ ID NO: 249 - DNA, 27 bp, Homo sapiens
  source 1..27: /mol_type="other DNA" /organism="Homo sapiens"
ctgagcccgcccccacccagtgcaaaa

SEQ ID NO: 250 - DNA, 27 bp, Homo sapiens
  source 1..27: /mol_type="other DNA" /organism="Homo sapiens"
tctgtgaaagtttctgttctctctctc

SEQ ID NO: 251 - DNA, 26 bp, Homo sapiens
  source 1..26: /mol_type="other DNA" /organism="Homo sapiens"
agaagcttgagcaaaggccttgagat

SEQ ID NO: 252 - DNA, 21 bp, Homo sapiens
  source 1..21: /mol_type="other DNA" /organism="Homo sapiens"
ctaaagggcaggtgccagctg

SEQ ID NO: 253 - DNA, 27 bp, Homo sapiens
  source 1..27: /mol_type="other DNA" /organism="Homo sapiens"
tcttctcttagaaggacactggtcaga

SEQ ID NO: 254 - DNA, 27 bp, Homo sapiens
  source 1..27: /mol_type="other DNA" /organism="Homo sapiens"
ccataatagaagggtgcacgggaattt

SEQ ID NO: 255 - DNA, 27 bp, Homo sapiens
  source 1..27: /mol_type="other DNA" /organism="Homo sapiens"
gccggggactttgactattaaatgaac

SEQ ID NO: 256 - DNA, 21 bp, Homo sapiens
  source 1..21: /mol_type="other DNA" /organism="Homo sapiens"
caggtaccttcctgacgccca

SEQ ID NO: 257 - DNA, 28 bp, Homo sapiens
  source 1..28: /mol_type="other DNA" /organism="Homo sapiens"
gctgtttaagggtaaaggggtagttact

SEQ ID NO: 258 - DNA, 27 bp, Homo sapiens
  source 1..27: /mol_type="other DNA" /organism="Homo sapiens"
ggagtagctttcaattattttggagcc

SEQ ID NO: 259 - DNA, 27 bp, Homo sapiens
  source 1..27: /mol_type="other DNA" /organism="Homo sapiens"
gacttaatacagacgatggcatgggct

SEQ ID NO: 260 - DNA, 27 bp, Homo sapiens
  source 1..27: /mol_type="other DNA" /organism="Homo sapiens"
gagtgcatagctctcatggaaaaagtc

SEQ ID NO: 261 - DNA, 25 bp, Homo sapiens
  source 1..25: /mol_type="other DNA" /organism="Homo sapiens"
atgacaatgatcttagggccacgag

SEQ ID NO: 262 - DNA, 23 bp, Homo sapiens
  source 1..23: /mol_type="other DNA" /organism="Homo sapiens"
tagtcgagggaggctgctctcag

SEQ ID NO: 263 - DNA, 21 bp, Homo sapiens
  source 1..21: /mol_type="other DNA" /organism="Homo sapiens"
ctttgtccctcaggcttggcc

SEQ ID NO: 264 - DNA, 26 bp, Homo sapiens
  source 1..26: /mol_type="other DNA" /organism="Homo sapiens"
aagaggataggctaactgactgcctt

SEQ ID NO: 265 - DNA, 27 bp, Homo sapiens
  source 1..27: /mol_type="other DNA" /organism="Homo sapiens"
cagtttgcactaaatgattacaggtta

SEQ ID NO: 266 - DNA, 29 bp, Homo sapiens
  source 1..29: /mol_type="other DNA" /organism="Homo sapiens"
ataaacactaacatgtaacattgctagag

SEQ ID NO: 267 - DNA, 29 bp, Homo sapiens
  source 1..29: /mol_type="other DNA" /organism="Homo sapiens"
acagtctccagagtatattagcttagttc

SEQ ID NO: 268 - DNA, 29 bp, Homo sapiens
  source 1..29: /mol_type="other DNA" /organism="Homo sapiens"
cattcatgaacttagttggcaattaaatt

SEQ ID NO: 269 - DNA, 27 bp, Homo sapiens
  source 1..27: /mol_type="other DNA" /organism="Homo sapiens"
cgagctcaattttcttgtccctgcttt

SEQ ID NO: 270 - DNA, 25 bp, Homo sapiens
  source 1..25: /mol_type="other DNA" /organism="Homo sapiens"
acttactgttgtgtgcagtccaagc